European Patent Application EP 4 692 360 A1, published February 11, 2026. Title: EXPRESSION VECTOR AND COMPOSITION FOR TREATING NERVOUS SYSTEM DISEASES. Applicant: SHANGHAI GENEMAGIC BIOSCIENCES CO., LTD. The sequence listing filed with the application follows.

SEQUENCE LISTING (95 sequences)

SEQ ID NO: 1 - protein, 1097 aa, synthetic construct
MATQVMGQSSGGGGLFTSSGNIGMALPNDMYDLHDLSKAELAAPQLIMLANVALTGEVNGSCCDYLVGEERQMAELMPVGDNNFSDSEEGEGLEESADIKGEPHGLENMELRSLELSVVEPQPVFEASGAPDIYSSNKDLPPETPGAEDKGKSSKTKPFRCKPCQYEAESEEQFVHHIRVHSAKKFFVEESAEKQAKARESGSSTAEEGDFSKGPIRCDRCGYNTNRYDHYTAHLKHHTRAGDNERVYKCIICTYTTVSEYHWRKHLRNHFPRKVYTCGKCNYFSDRKNNYVQHVRTHTGERPYKCELCPYSSSQKTHLTRHMRTHSGEKPFKCDQCSYVASNQHEVTRHARQVHNGPKPLNCPHCDYKTADRSNFKKHVELHVNPRQFNCPVCDYAASKKCNLQYHFKSKHPTCPNKTMDVSKVKLKKTKKREADLPDNITNEKTEIEQTKIKGDVAGKKNEKSVKAEKRDVSKEKKPSNNVSVIQVTTRTRKSVTEVKEMDVHTGSNSEKFSKTKKSKRKLEVDSHSLHGPVNDEESSTKKKKKVESKSKNNSQEVPKGDSKVEENKKQNTCMKKSTKKKTLKNKSSKKSSKPPQKEPVEKGSAQMDPPQMGPAPTEAVQKGPVQVEPPPPMEHAQMEGAQIRPAPDEPVQMEVVQEGPAQKELLPPVEPAQMVGAQIVLAHMELPPPMETAQTEVAQMGPAPMEPAQMEVAQVESAPMQVVQKEPVQMELSPPMEVVQKEPVQIELSPPMEVVQKEPVKIELSPPIEVVQKEPVQMELSPPMGVVQKEPAQREPPPPREPPLHMEPISKKPPLRKDKKEKSNMQSERARKEQVLIEVGLVPVKDSWLLKESVSTEDLSPPSPPLPKENLREEASGDQKLLNTGEGNKEAPLQKVGAEEADESLPGLAANINESTHISSSGQNLNTPEGETLNGKHQTDSIVCEMKMDTDQNTRENLTGINSTVEEPVSPMLPPSAVEEREAVSKTALASPPATMAANESQEIDEDEGIHSHEGSDLSDNMSEGSDDSGLHGARPVPQESSRKNAKEALAVKAAKGDFVCIFCDRSFRKGKDYSKHLNRHLVNVYYLEEAAQGQE

SEQ ID NO: 2 - protein, 254 aa, synthetic construct
FRCKPCQYEAESEEQFVHHIRVHSAKKFFVEESAEKQAKARESGSSTAEEGDFSKGPIRCDRCGYNTNRYDHYTAHLKHHTRAGDNERVYKCIICTYTTVSEYHWRKHLRNHFPRKVYTCGKCNYFSDRKNNYVQHVRTHTGERPYKCELCPYSSSQKTHLTRHMRTHSGEKPFKCDQCSYVASNQHEVTRHARQVHNGPKPLNCPHCDYKTADRSNFKKHVELHVNPRQFNCPVCDYAASKKCNLQYHFKSKH

SEQ ID NO: 3 - protein, 23 aa, synthetic construct
FRCKPCQYEAESEEQFVHHIRVH

SEQ ID NO: 4 - protein, 32 aa, synthetic construct
IRCDRCGYNTNRYDHYTAHLKHHTRAGDNERV

SEQ ID NO: 5 - protein, 19 aa, synthetic construct
YKCIICTYTTVSEYHWRKH

SEQ ID NO: 6 - protein, 23 aa, synthetic construct
YTCGKCNYFSDRKNNYVQHVRTH

SEQ ID NO: 7 - protein, 28 aa, synthetic construct
YKCELCPYSSSQKTHLTRHMRTHSGEKP

SEQ ID NO: 8 - protein, 29 aa, synthetic construct
FKCDQCSYVASNQHEVTRHARQVHNGPKP

SEQ ID NO: 9 - protein, 28 aa, synthetic construct
LNCPHCDYKTADRSNFKKHVELHVNPRQ

SEQ ID NO: 10 - protein, 24 aa, synthetic construct
FNCPVCDYAASKKCNLQYHFKSKH

SEQ ID NO: 11 - protein, 66 aa, synthetic construct
DLSHPPPRGHLDELTTTLESMTEDLNLDSPLTPELNEILDTFLNDECLLHAMHISTGLSIFDTSLF

SEQ ID NO: 12 - protein, 112 aa, synthetic construct
MATQVMGQSSGGGGLFTSSGNIGMALPNDMYDLHDLSKAELAAPQLIMLANVALTGEVNGSCCDYLVGEERQMAELMPVGDNNFSDSEEGEGLEESADIKGEPHGLENMELR

SEQ ID NO: 13 - protein, 90 aa, synthetic construct
DEGIHSHEGSDLSDNMSEGSDDSGLHGARPVPQESSRKNAKEALAVKAAKGDFVCIFCDRSFRKGKDYSKHLNRHLVNVYYLEEAAQGQE

SEQ ID NO: 14 - protein, 265 aa, synthetic construct
KTKPFRCKPCQYEAESEEQFVHHIRVHSAKKFFVEESAEKQAKARESGSSTAEEGDFSKGPIRCDRCGYNTNRYDHYTAHLKHHTRAGDNERVYKCIICTYTTVSEYHWRKHLRNHFPRKVYTCGKCNYFSDRKNNYVQHVRTHTGERPYKCELCPYSSSQKTHLTRHMRTHSGEKPFKCDQCSYVASNQHEVTRHARQVHNGPKPLNCPHCDYKTADRSNFKKHVELHVNPRQFNCPVCDYAASKKCNLQYHFKSKHPTCPNKT

SEQ ID NO: 15 - DNA, 795 bp, synthetic construct
  source 1..795: mol_type = other DNA
aagaccaaaccctttcgctgtaagccatgccaatatgaagcagaatctgaagaacagtttgtgcatcacatcagagttcacagtgctaagaaattttttgtggaagagagtgcagagaagcaggcaaaagccagggaatctggctcttccactgcagaagagggagatttctccaagggccccattcgctgtgaccgctgcggctacaatactaatcgatatgatcactatacagcacacctgaaacaccacaccagagctggggataatgagcgagtctacaagtgtatcatttgcacatacacaacagtgagcgagtatcactggaggaaacatttaagaaaccattttccaaggaaagtatacacatgtggaaaatgcaactatttttcagacagaaaaaacaattatgttcagcatgttagaactcatacaggagaacgcccatataaatgtgaactttgtccttactcaagttctcagaagactcatctaactagacatatgcgtactcattcaggtgagaagccatttaaatgtgatcagtgcagttatgtggcctctaatcaacatgaagtaacccgccatgcaagacaggttcacaatgggcctaaacctcttaattgcccacactgtgattacaaaacagcagatagaagcaacttcaaaaaacatgtagagctacatgtgaacccacggcagttcaattgccctgtatgtgactatgcagcttccaagaagtgtaatctacagtatcacttcaaatctaagcatcctacttgtcctaataaaaca

SEQ ID NO: 16 - DNA, 298 bp, synthetic construct
  source 1..298: mol_type = other DNA
ataacttacggtaaatggcccgcctggctgaccgcccaacgacccccgcccattgacgtcaataatgacgtatgttcccatagtaacgccaatagggactttccattgacgtcaatgggtggagtatttacggtaaactgcccacttggcagtacatcaagtgtatcatatgccaagtacgccccctattgacgtcaatgacggtaaatggcccgcctggcattatgcccagtacatgaccttatgggactttcctacttggcagtacatctacgtattagtcatcgctattaccatg

SEQ ID NO: 17 - DNA, 97 bp, synthetic construct
  source 1..97: mol_type = other DNA
gtaagtttagtctttttgtcttttatttcaggtcccggatccggtggtggtgcaaatcaaagaactgctcctcagtggatgttgcctttacttctag

SEQ ID NO: 18 - DNA, 92 bp, synthetic construct
  source 1..92: mol_type = other DNA
aagaggtaagggtttaagggatggttggttggtggggtattaatgtttaattacctggagcacctgcctgaaatcactttttttcaggttgg

SEQ ID NO: 19 - DNA, 573 bp, synthetic construct
  source 1..573: mol_type = other DNA
gtgagtttggggacccttgattgttctttctttttcgctattgtaaaattcatgttatatggagggggcaaagttttcagggtgttgtttagaatgggaagatgtcccttgtatcaccatggaccctcatgataattttgtttctttcactttctactctgttgacaaccattgtctcctcttattttcttttcattttctgtaactttttcgttaaactttagcttgcatttgtaacgaatttttaaattcacttttgtttatttgtcagattgtaagtactttctctaatcacttttttttcaaggcaatcagggtatattatattgtacttcagcacagttttagagaacaattgttataattaaatgataaggtagaatatttctgcatataaattctggctggcgtggaaatattcttattggtagaaacaactacaccctggtcatcatcctgcctttctctttatggttacaatgatatacactgtttgagatgaggataaaatactctgagtccaaaccgggcccctctgctaaccatgttcatgccttcttctctttcctacag

SEQ ID NO: 20 - DNA, 99 bp, synthetic construct
  source 1..99: mol_type = other DNA
gtaagtgagtcatatactcctagcagtcttcaatgtgaacgactttggaacaagcgttcgcacggcacattactaaccaggctctttcctcttcttcag

SEQ ID NO: 21 - DNA, 99 bp, synthetic construct
  source 1..99: mol_type = other DNA
gtaagtggatcaacagcatctagttgtcttctgcaaccatcactccttactgaactcacgctcgcggctctactaacgcgaccttccttctccctccag

SEQ ID NO: 22 - DNA, 99 bp, synthetic construct
  source 1..99: mol_type = other DNA
gtaagtatcactcaactatctagccgtcttcgggacgtcatcacatccagtcaaccgtgggctacgcatctactaacagcgtccttccttctttctcag

SEQ ID NO: 23 - DNA, 10 bp, synthetic construct
  source 1..10: mol_type = other DNA
gccrccatgg

SEQ ID NO: 24 - protein, 18 aa, synthetic construct
KRTADGSEFESPKKKRKV

SEQ ID NO: 25 - DNA, 54 bp, synthetic construct
  source 1..54: mol_type = other DNA
aaacggacagccgatggcagcgagttcgagagccccaagaagaagagaaaggtg

SEQ ID NO: 26 - protein, 55 aa, synthetic construct
RADALDDFDLDMLGSDALDDFDLDMLGSDALDDFDLDMLGSDALDDFDLDMLYID

SEQ ID NO: 27 - DNA, 165 bp, synthetic construct
  source 1..165: mol_type = other DNA
agagccgacgctctggacgacttcgacctggatatgctgggctccgatgctctggatgacttcgacctggacatgctgggcagcgacgccctggacgacttcgacctggacatgctgggaagcgacgccctggatgattttgatctggacatgctctacatcgac

SEQ ID NO: 28 - protein, 313 aa, synthetic construct
PSGQISNQALALAPSSAPVLAQTMVPSSAMVPLAQPPAPAPVLTPGPPQSLSAPVPKSTQAGEGTLSEALLHLQFDADEDLGALLGNSTDPGVFTDLASVDNSEFQQLLNQGVSMSHSTAEPMLMEYPEAITRLVTGSQRPPDPAPTPLGTSGLPNGLSGDEDFSSIADMDFSALLSQISSSGQGGGGSGFSVDTSALLDLFSPSVTVPDMSLPDLDSSLASIQELLSPQEPPRPPEAENSSPDSGKQLVHYTAQPLFLLDPGSVDTGSNDLPVLFELGEGSYFSEGDGFAEDPTISLLTGSEPPKAKDPTVS

SEQ ID NO: 29 - DNA, 939 bp, synthetic construct
  source 1..939: mol_type = other DNA
ccttcagggcagatcagcaaccaggccctggctctggcccctagctccgctccagtgctggcccagactatggtgccctctagtgctatggtgcctctggcccagccacctgctccagcccctgtgctgaccccaggaccaccccagtcactgagcgctccagtgcccaagtctacacaggccggcgaggggactctgagtgaagctctgctgcacctgcagttcgacgctgatgaggacctgggagctctgctggggaacagcaccgatcccggagtgttcacagatctggcctccgtggacaactctgagtttcagcagctgctgaatcagggcgtgtccatgtctcatagtacagccgaaccaatgctgatggagtaccccgaagccattacccggctggtgaccggcagccagcggccccccgaccccgctccaactcccctgggaaccagcggcctgcctaatgggctgtccggagatgaagacttctcaagcatcgctgatatggactttagtgccctgctgtcacagatttcctctagtgggcagggaggaggtggaagcggcttcagcgtggacaccagtgccctgctggacctgttcagcccctcggtgaccgtgcccgacatgagcctgcctgaccttgacagcagcctggccagtatccaagagctcctgtctccccaggagccccccaggcctcccgaggcagagaacagcagcccggattcagggaagcagctggtgcactacacagcgcagccgctgttcctgctggaccccggctccgtggacaccgggagcaacgacctgccggtgctgtttgagctgggagagggctcctacttctccgaaggggacggcttcgccgaggaccccaccatctccctgctgacaggctcggagcctcccaaagccaaggaccccactgtctcc

SEQ ID NO: 30 - protein, 308 aa, synthetic construct
MKRTADGSEFESPKKKRKVGSGKTKPFRCKPCQYEAESEEQFVHHIRVHSAKKFFVEESAEKQAKARESGSSTAEEGDFSKGPIRCDRCGYNTNRYDHYTAHLKHHTRAGDNERVYKCIICTYTTVSEYHWRKHLRNHFPRKVYTCGKCNYFSDRKNNYVQHVRTHTGERPYKCELCPYSSSQKTHLTRHMRTHSGEKPFKCDQCSYVASNQHEVTRHARQVHNGPKPLNCPHCDYKTADRSNFKKHVELHVNPRQFNCPVCDYAASKKCNLQYHFKSKHPTCPNKTMGSKRTADGSEFESPKKKRKV

SEQ ID NO: 31 - DNA, 924 bp, synthetic construct
  source 1..924: mol_type = other DNA
atgaaacggacagccgatggcagcgagttcgagagccccaagaagaagagaaaggtgggcagcggcaagaccaagcccttcaggtgtaaaccctgccagtacgaggccgagtctgaggaacagtttgtccaccacatcagagtgcacagcgctaagaaattcttcgttgaggaatctgccgagaagcaggccaaggcccgggaaagcggctccagtacagccgaagagggcgacttcagcaagggccctatccggtgcgacagatgtggctataataccaacagatacgaccactacacagcgcacctgaagcaccacacccgggccggcgacaacgagagagtgtacaagtgcatcatctgcacctacaccacagtgtccgagtaccactggcggaaacatctcagaaaccactttccaagaaaggtgtacacctgcggcaagtgcaactacttcagcgaccggaagaacaactacgtgcagcacgtgcggacacacaccggcgagagaccttataagtgtgaactgtgcccttacagcagcagccagaaaactcacctgacccgccacatgagaacccatagcggagaaaagccatttaagtgcgaccagtgcagctacgtggccagcaatcaacacgaggtgaccagacacgccagacaggtgcacaacggccctaagcctctgaactgtccccactgcgactacaaaaccgccgatcggagcaacttcaagaaacacgtggaactgcacgtgaatcctagacagttcaactgccccgtgtgcgattacgccgcctccaagaagtgtaacctgcaataccacttcaagagcaagcatcctacatgccctaacaagaccatgggcagcaagagaacagctgatggcagcgaattcgagtcccctaagaaaaaaagaaaggtc

SEQ ID NO: 32 - protein, 475 aa, synthetic construct
MRADALDDFDLDMLGSDALDDFDLDMLGSDALDDFDLDMLGSDALDDFDLDMLYIDGSGSGGSGSGSGGSGSGGSGSGKRTADGSEFESPKKKRKVGSGKTKPFRCKPCQYEAESEEQFVHHIRVHSAKKFFVEESAEKQAKARESGSSTAEEGDFSKGPIRCDRCGYNTNRYDHYTAHLKHHTRAGDNERVYKCIICTYTTVSEYHWRKHLRNHFPRKVYTCGKCNYFSDRKNNYVQHVRTHTGERPYKCELCPYSSSQKTHLTRHMRTHSGEKPFKCDQCSYVASNQHEVTRHARQVHNGPKPLNCPHCDYKTADRSNFKKHVELHVNPRQFNCPVCDYAASKKCNLQYHFKSKHPTCPNKTMGSKRTADGSEFESPKKKRKVSGGSSGGSSGSETPGTSESATPESSGGSSGGSSRADALDDFDLDMLGSDALDDFDLDMLGSDALDDFDLDMLGSDALDDFDLDMLYIDGS

SEQ ID NO: 33 - DNA, 1425 bp, synthetic construct
  source 1..1425: mol_type = other DNA
atgagagccgacgccctggatgacttcgacctggacatgctcggcagcgacgccctggacgacttcgacctggatatgctgggctccgatgctctggacgacttcgacctggacatgctgggctctgatgccctggatgattttgatctggacatgctgtacatcgacggcagcggcagcggcggcagcggcagcggcagcggcggaagcggatctggaggcagcggaagcggcaaacggacagccgatggcagcgagttcgagagccccaagaagaagagaaaggtgggcagcggcaagaccaagcccttcaggtgtaaaccctgccagtacgaggccgagtctgaggaacagtttgtccaccacatcagagtgcacagcgctaagaaattcttcgttgaggaatctgccgagaagcaggccaaggcccgggaaagcggctccagtacagccgaagagggcgacttcagcaagggccctatccggtgcgacagatgtggctataataccaacagatacgaccactacacagcgcacctgaagcaccacacccgggccggcgacaacgagagagtgtacaagtgcatcatctgcacctacaccacagtgtccgagtaccactggcggaaacatctcagaaaccactttccaagaaaggtgtacacctgcggcaagtgcaactacttcagcgaccggaagaacaactacgtgcagcacgtgcggacacacaccggcgagagaccttataagtgtgaactgtgcccttacagcagcagccagaaaactcacctgacccgccacatgagaacccatagcggagaaaagccatttaagtgcgaccagtgcagctacgtggccagcaatcaacacgaggtgaccagacacgccagacaggtgcacaacggccctaagcctctgaactgtccccactgcgactacaaaaccgccgatcggagcaacttcaagaaacacgtggaactgcacgtgaatcctagacagttcaactgccccgtgtgcgattacgccgcctccaagaagtgtaacctgcaataccacttcaagagcaagcatcctacatgccctaacaagaccatgggcagcaagcggaccgccgatggctctgagttcgagagccccaagaagaaaagaaaggtgtccggcggcagcagcggaggcagcagcggcagcgagacacctggcaccagcgaatccgccacccctgagagcagcggcggctcttctggcggaagctctagagccgacgctctggacgacttcgacctggatatgctgggctccgatgctctggatgacttcgacctggacatgctgggcagcgacgccctggacgacttcgacctggacatgctgggaagcgacgccctggatgattttgatctggacatgctctacatcgacggcagc

SEQ ID NO: 34 - protein, 801 aa, synthetic construct
MRADALDDFDLDMLGSDALDDFDLDMLGSDALDDFDLDMLGSDALDDFDLDMLYIDGSGSGGSGSGSGGSGSGGSGSGKRTADGSEFESPKKKRKVGSGKTKPFRCKPCQYEAESEEQFVHHIRVHSAKKFFVEESAEKQAKARESGSSTAEEGDFSKGPIRCDRCGYNTNRYDHYTAHLKHHTRAGDNERVYKCIICTYTTVSEYHWRKHLRNHFPRKVYTCGKCNYFSDRKNNYVQHVRTHTGERPYKCELCPYSSSQKTHLTRHMRTHSGEKPFKCDQCSYVASNQHEVTRHARQVHNGPKPLNCPHCDYKTADRSNFKKHVELHVNPRQFNCPVCDYAASKKCNLQYHFKSKHPTCPNKTMGSKRTADGSEFESPKKKRKVSGGSSGGSSGSETPGTSESATPESSGGSSGGSSRADALDDFDLDMLGSDALDDFDLDMLGSDALDDFDLDMLGSDALDDFDLDMLYIDGSDGSGGGGSGGGGSPSGQISNQALALAPSSAPVLAQTMVPSSAMVPLAQPPAPAPVLTPGPPQSLSAPVPKSTQAGEGTLSEALLHLQFDADEDLGALLGNSTDPGVFTDLASVDNSEFQQLLNQGVSMSHSTAEPMLMEYPEAITRLVTGSQRPPDPAPTPLGTSGLPNGLSGDEDFSSIADMDFSALLSQISSSGQGGGGSGFSVDTSALLDLFSPSVTVPDMSLPDLDSSLASIQELLSPQEPPRPPEAENSSPDSGKQLVHYTAQPLFLLDPGSVDTGSNDLPVLFELGEGSYFSEGDGFAEDPTISLLTGSEPPKAKDPTVS

SEQ ID NO: 35 - DNA, 2403 bp, synthetic construct
  source 1..2403: mol_type = other DNA
atgagagccgacgccctggatgacttcgacctggacatgctcggcagcgacgccctggacgacttcgacctggatatgctgggctccgatgctctggacgacttcgacctggacatgctgggctctgatgccctggatgattttgatctggacatgctgtacatcgacggcagcggcagcggcggcagcggcagcggcagcggcggaagcggatctggaggcagcggaagcggcaaacggacagccgatggcagcgagttcgagagccccaagaagaagagaaaggtgggcagcggcaagaccaagcccttcaggtgtaaaccctgccagtacgaggccgagtctgaggaacagtttgtccaccacatcagagtgcacagcgctaagaaattcttcgttgaggaatctgccgagaagcaggccaaggcccgggaaagcggctccagtacagccgaagagggcgacttcagcaagggccctatccggtgcgacagatgtggctataataccaacagatacgaccactacacagcgcacctgaagcaccacacccgggccggcgacaacgagagagtgtacaagtgcatcatctgcacctacaccacagtgtccgagtaccactggcggaaacatctcagaaaccactttccaagaaaggtgtacacctgcggcaagtgcaactacttcagcgaccggaagaacaactacgtgcagcacgtgcggacacacaccggcgagagaccttataagtgtgaactgtgcccttacagcagcagccagaaaactcacctgacccgccacatgagaacccatagcggagaaaagccatttaagtgcgaccagtgcagctacgtggccagcaatcaacacgaggtgaccagacacgccagacaggtgcacaacggccctaagcctctgaactgtccccactgcgactacaaaaccgccgatcggagcaacttcaagaaacacgtggaactgcacgtgaatcctagacagttcaactgccccgtgtgcgattacgccgcctccaagaagtgtaacctgcaataccacttcaagagcaagcatcctacatgccctaacaagaccatgggcagcaagcggaccgccgatggctctgagttcgagagccccaagaagaaaagaaaggtgtccggcggcagcagcggaggcagcagcggcagcgagacacctggcaccagcgaatccgccacccctgagagcagcggcggctcttctggcggaagctctagagccgacgctctggacgacttcgacctggatatgctgggctccgatgctctggatgacttcgacctggacatgctgggcagcgacgccctggacgacttcgacctggacatgctgggaagcgacgccctggatgattttgatctggacatgctctacatcgacggcagcgatggtagtggcggtggtggttcaggaggcggcggaagcccttcagggcagatcagcaaccaggccctggctctggcccctagctccgctccagtgctggcccagactatggtgccctctagtgctatggtgcctctggcccagccacctgctccagcccctgtgctgaccccaggaccaccccagtcactgagcgctccagtgcccaagtctacacaggccggcgaggggactctgagtgaagctctgctgcacctgcagttcgacgctgatgaggacctgggagctctgctggggaacagcaccgatcccggagtgttcacagatctggcctccgtggacaactctgagtttcagcagctgctgaatcagggcgtgtccatgtctcatagtacagccgaaccaatgctgatggagtaccccgaagccattacccggctggtgaccggcagccagcggccccccgaccccgctccaactcccctgggaaccagcggcctgcctaatgggctgtccggagatgaagacttctcaagcatcgctgatatggactttagtgccctgctgtcacagatttcctctagtgggcagggaggaggtggaagcggcttcagcgtggacaccagtgccctgctggacctgttcagcccctcggtgaccgtgcccgacatgagcctgcctgaccttgacagcagcctggccagtatccaagagctcctgtctccccaggagccccccaggcctcccgaggcagagaacagcagcccggattcagggaagcagctggtgcactacacagcgcagccgctgttcctgctggaccccggctccgtggacaccgggagcaacgacctgccggtgctgtttgagctgggagagggctcctacttctccgaaggggacggcttcgccgaggaccccaccatctccctgctgacaggctcggagcctcccaaagccaaggaccccactgtctcc

SEQ ID NO: 36 - DNA, 2995 bp, synthetic construct
  source 1..2995: mol_type = other DNA
ataacttacggtaaatggcccgcctggctgaccgcccaacgacccccgcccattgacgtcaataatgacgtatgttcccatagtaacgccaatagggactttccattgacgtcaatgggtggagtatttacggtaaactgcccacttggcagtacatcaagtgtatcatatgccaagtacgccccctattgacgtcaatgacggtaaatggcccgcctggcattatgcccagtacatgaccttatgggactttcctacttggcagtacatctacgtattagtcatcgctattaccatgctcgagtactagaacatatcctggtgtggagtaggggacgctgctctgacagaggctcgggggcctgagctggctctgtgagctggggaggaggcagacagccaggccttgtctgcaagcagacctggcagcattgggctggccgccccccagggcctcctcttcatgcccagtgaatgactcaccttggcacagacacaatgttcggggtgggcacagtgcctgcttcccgccgcaccccagcccccctcaaatgccttccgagaagcccattgagcagggggcttgcattgcaccccagcctgacagcctggcatcttgggataaaagcagcacagccccctaggggctgcccttgctgtgtggcgccaccggcggtggagaacaaggctctattcagcctgtgcccaggaaaggggatcaggggatgcccaggcatggacagtgggtggcagggggggagaggagggctgtctgcttcccagaagtccaaggacacaaatgggtgaggggagagctctccccatagctgggctgcggcccaaccccaccccctcaggctatgccagggggtgttgccaggggcacccgggcatcgccagtctagcccactccttcataaagccctcgcatcccaggagcgagcagagccagagcaggttggagaggagacgcatcacctccgctgctcgcgaattggatcaagaggtaagggtttaagggatggttggttggtggggtattaatgtttaattacctggagcacctgcctgaaatcactttttttcaggttggggatccgccaccatgagagccgacgccctggatgacttcgacctggacatgctcggcagcgacgccctggacgacttcgacctggatatgctgggctccgatgctctggacgacttcgacctggacatgctgggctctgatgccctggatgattttgatctggacatgctgtacatcgacggcagcggcagcggcggcagcggcagcggcagcggcggaagcggatctggaggcagcggaagcggcaaacggacagccgatggcagcgagttcgagagccccaagaagaagagaaaggtgggcagcggcaagaccaagcccttcaggtgtaaaccctgccagtacgaggccgagtctgaggaacagtttgtccaccacatcagagtgcacagcgctaagaaattcttcgttgaggaatctgccgagaagcaggccaaggcccgggaaagcggctccagtacagccgaagagggcgacttcagcaagggccctatccggtgcgacagatgtggctataataccaacagatacgaccactacacagcgcacctgaagcaccacacccgggccggcgacaacgagagagtgtacaagtgcatcatctgcacctacaccacagtgtccgagtaccactggcggaaacatctcagaaaccactttccaagaaaggtgtacacctgcggcaagtgcaactacttcagcgaccggaagaacaactacgtgcagcacgtgcggacacacaccggcgagagaccttataagtgtgaactgtgcccttacagcagcagccagaaaactcacctgacccgccacatgagaacccatagcggagaaaagccatttaagtgcgaccagtgcagctacgtggccagcaatcaacacgaggtgaccagacacgccagacaggtgcacaacggccctaagcctctgaactgtccccactgcgactacaaaaccgccgatcggagcaacttcaagaaacacgtggaactgcacgtgaatcctagacagttcaactgccccgtgtgcgattacgccgcctccaagaagtgtaacctgcaataccacttcaagagcaagcatcctacatgccctaacaagaccatgggcagcaagcggaccgccgatggctctgagttcgagagccccaagaagaaaagaaaggtgtccggcggcagcagcggaggcagcagcggcagcgagacacctggcaccagcgaatccgccacccctgagagcagcggcggctcttctggcggaagctctagagccgacgctctggacgacttcgacctggatatgctgggctccgatgctctggatgacttcgacctggacatgctgggcagcgacgccctggacgacttcgacctggacatgctgggaagcgacgccctggatgattttgatctggacatgctctacatcgacggcagcgatatcgactacaaggatgacgacgacaagtaaaattcataatcaacctctggattacaaaatttgtgaaagattgactggtattcttaactatgttgctccttttacgctatgtggatacgctgctttaatgcctttgtatcatgctattgcttcccgtatggctttcattttctcctccttgtataaatcctggttagttcttgccacggcggaactcatcgccgcctgccttgcccgctgctggacaggggctcggctgttgggcactgacaattccgtggtgtttatttgtgaaatttgtgatgctattgctttatttgtaaccatctagctttatttgtgaaatttgtgatgctattgctttatttgtaaccattataagctgcaataaacaagttaacaacaacaattgcattcattttatgtttcaggttcagggggagatgtgggaggttttttaaa

SEQ ID NO: 37 - DNA, 3970 bp, synthetic construct
  source 1..3970: mol_type = other DNA
ataacttacggtaaatggcccgcctggctgaccgcccaacgacccccgcccattgacgtcaataatgacgtatgttcccatagtaacgccaatagggactttccattgacgtcaatgggtggagtatttacggtaaactgcccacttggcagtacatcaagtgtatcatatgccaagtacgccccctattgacgtcaatgacggtaaatggcccgcctggcattatgcccagtacatgaccttatgggactttcctacttggcagtacatctacgtattagtcatcgctattaccatgctcgagtactagaacatatcctggtgtggagtaggggacgctgctctgacagaggctcgggggcctgagctggctctgtgagctggggaggaggcagacagccaggccttgtctgcaagcagacctggcagcattgggctggccgccccccagggcctcctcttcatgcccagtgaatgactcaccttggcacagacacaatgttcggggtgggcacagtgcctgcttcccgccgcaccccagcccccctcaaatgccttccgagaagcccattgagcagggggcttgcattgcaccccagcctgacagcctggcatcttgggataaaagcagcacagccccctaggggctgcccttgctgtgtggcgccaccggcggtggagaacaaggctctattcagcctgtgcccaggaaaggggatcaggggatgcccaggcatggacagtgggtggcagggggggagaggagggctgtctgcttcccagaagtccaaggacacaaatgggtgaggggagagctctccccatagctgggctgcggcccaaccccaccccctcaggctatgccagggggtgttgccaggggcacccgggcatcgccagtctagcccactccttcataaagccctcgcatcccaggagcgagcagagccagagcaggttggagaggagacgcatcacctccgctgctcgcgaattggatcaagaggtaagggtttaagggatggttggttggtggggtattaatgtttaattacctggagcacctgcctgaaatcactttttttcaggttggggatccgccaccatgagagccgacgccctggatgacttcgacctggacatgctcggcagcgacgccctggacgacttcgacctggatatgctgggctccgatgctctggacgacttcgacctggacatgctgggctctgatgccctggatgattttgatctggacatgctgtacatcgacggcagcggcagcggcggcagcggcagcggcagcggcggaagcggatctggaggcagcggaagcggcaaacggacagccgatggcagcgagttcgagagccccaagaagaagagaaaggtgggcagcggcaagaccaagcccttcaggtgtaaaccctgccagtacgaggccgagtctgaggaacagtttgtccaccacatcagagtgcacagcgctaagaaattcttcgttgaggaatctgccgagaagcaggccaaggcccgggaaagcggctccagtacagccgaagagggcgacttcagcaagggccctatccggtgcgacagatgtggctataataccaacagatacgaccactacacagcgcacctgaagcaccacacccgggccggcgacaacgagagagtgtacaagtgcatcatctgcacctacaccacagtgtccgagtaccactggcggaaacatctcagaaaccactttccaagaaaggtgtacacctgcggcaagtgcaactacttcagcgaccggaagaacaactacgtgcagcacgtgcggacacacaccggcgagagaccttataagtgtgaactgtgcccttacagcagcagccagaaaactcacctgacccgccacatgagaacccatagcggagaaaagccatttaagtgcgaccagtgcagctacgtggccagcaatcaacacgaggtgaccagacacgccagacaggtgcacaacggccctaagcctctgaactgtccccactgcgactacaaaaccgccgatcggagcaacttcaagaaacacgtggaactgcacgtgaatcctagacagttcaactgccccgtgtgcgattacgccgcctccaagaagtgtaacctgcaataccacttcaagagcaagcatcctacatgccctaacaagaccatgggcagcaagcggaccgccgatggctctgagttcgagagccccaagaagaaaagaaaggtgtccggcggcagcagcggaggcagcagcggcagcgagacacctggcaccagcgaatccgccacccctgagagcagcggcggctcttctggcggaagctctagagccgacgctctggacgacttcgacctggatatgctgggctccgatgctctggatgacttcgacctggacatgctgggcagcgacgccctggacgacttcgacctggacatgctgggaagcgacgccctggatgattttgatctggacatgctctacatcgacggcagcgatggtagtggcggtggtggttcaggaggcggcggaagcccttcagggcagatcagcaaccaggccctggctctggcccctagctccgctccagtgctggcccagactatggtgccctctagtgctatggtgcctctggcccagccacctgctccagcccctgtgctgaccccaggaccaccccagtcactgagcgctccagtgcccaagtctacacaggccggcgaggggactctgagtgaagctctgctgcacctgcagttcgacgctgatgaggacctgggagctctgctggggaacagcaccgatcccggagtgttcacagatctggcctccgtggacaactctgagtttcagcagctgctgaatcagggcgtgtccatgtctcatagtacagccgaaccaatgctgatggagtaccccgaagccattacccggctggtgaccggcagccagcggccccccgaccccgctccaactcccctgggaaccagcggcctgcctaatgggctgtccggagatgaagacttctcaagcatcgctgatatggactttagtgccctgctgtcacagatttcctctagtgggcagggaggaggtggaagcggcttcagcgtggacaccagtgccctgctggacctgttcagcccctcggtgaccgtgcccgacatgagcctgcctgaccttgacagcagcctggccagtatccaagagctcctgtctccccaggagccccccaggcctcccgaggcagagaacagcagcccggattcagggaagcagctggtgcactacacagcgcagccgctgttcctgctggaccccggctccgtggacaccgggagcaacgacctgccggtgctgtttgagctgggagagggctcctacttctccgaaggggacggcttcgccgaggaccccaccatctccctgctgacaggctcggagcctcccaaagccaaggaccccactgtctccatcgactacaaggatgacgacgacaagtaaaattcataatcaacctctggattacaaaatttgtgaaagattgactggtattcttaactatgttgctccttttacgctatgtggatacgctgctttaatgcctttgtatcatgctattgcttcccgtatggctttcattttctcctccttgtataaatcctggttagttcttgccacggcggaactcatcgccgcctgccttgcccgctgctggacaggggctcggctgttgggcactgacaattccgtggtgtttatttgtgaaatttgtgatgctattgctttatttgtaaccatctagctttatttgtgaaatttgtgatgctattgctttatttgtaaccattataagctgcaataaacaagttaacaacaacaattgcattcattttatgtttcaggttcagggggagatgtgggaggttttttaaa

SEQ ID NO: 38 - protein, 7 aa, synthetic construct
PKKKRKV

SEQ ID NO: 39 - protein, 16 aa, synthetic construct
KRPAATKKAGQAKKKK

SEQ ID NO: 40 - protein, 9 aa, synthetic construct
PAAKRVKLD

SEQ ID NO: 41 - protein, 11 aa, synthetic construct
RQRRNELKRSP

SEQ ID NO: 42 - protein, 38 aa, synthetic construct
NQSSNFGPMKGGNFGGRSSGPYGGGGQYFAKPRNQGGY

SEQ ID NO: 43 - protein, 42 aa, synthetic construct
RMRIZFKNKGKDTAELRRRRVEVSVELRKAKKDEQILKRRNV

SEQ ID NO: 44 - protein, 8 aa, synthetic construct
VSRKRPRP

SEQ ID NO: 45 - protein, 8 aa, synthetic construct
PPKKARED

SEQ ID NO: 46 - protein, 8 aa, synthetic construct
POPKKKPL

SEQ ID NO: 47 - protein, 12 aa, synthetic construct
SALIKKKKKMAP

SEQ ID NO: 48 - protein, 5 aa, synthetic construct
DRLRR

SEQ ID NO: 49 - protein, 7 aa, synthetic construct
PKQKKRK

SEQ ID NO: 50 - protein, 10 aa, synthetic construct
RKLKKKIKKL

SEQ ID NO: 51 - protein, 10 aa, synthetic construct
REKKKFLKRR

SEQ ID NO: 52 - protein, 20 aa, synthetic construct
KRKGDEVDGVDEVAKKKSKK

SEQ ID NO: 53 - protein, 17 aa, synthetic construct
RKCLQAGMNLEARKTKK

SEQ ID NO: 54 - protein, 11 aa, synthetic construct
LYPERLRRILT

SEQ ID NO: 55 - protein, 7 aa, synthetic construct
PKKKRKV

SEQ ID NO: 56 - DNA, 828 bp, synthetic construct
  source 1..828: mol_type = other DNA
atgcctaaaaagaaaagaaaggtgggttctggtaagaccaaaccctttcgctgtaagccatgccaatatgaagcagaatctgaagaacagtttgtgcatcacatcagagttcacagtgctaagaaattttttgtggaagagagtgcagagaagcaggcaaaagccagggaatctggctcttccactgcagaagagggagatttctccaagggccccattcgctgtgaccgctgcggctacaatactaatcgatatgatcactatacagcacacctgaaacaccacaccagagctggggataatgagcgagtctacaagtgtatcatttgcacatacacaacagtgagcgagtatcactggaggaaacatttaagaaaccattttccaaggaaagtatacacatgtggaaaatgcaactatttttcagacagaaaaaacaattatgttcagcatgttagaactcatacaggagaacgcccatataaatgtgaactttgtccttactcaagttctcagaagactcatctaactagacatatgcgtactcattcaggtgagaagccatttaaatgtgatcagtgcagttatgtggcctctaatcaacatgaagtaacccgccatgcaagacaggttcacaatgggcctaaacctcttaattgcccacactgtgattacaaaacagcagatagaagcaacttcaaaaaacatgtagagctacatgtgaacccacggcagttcaattgccctgtatgtgactatgcagcttccaagaagtgtaatctacagtatcacttcaaatctaagcatcctacttgtcctaataaaaca

SEQ ID NO: 57 - protein, 276 aa, synthetic construct
MPKKKRKVGSGKTKPFRCKPCQYEAESEEQFVHHIRVHSAKKFFVEESAEKQAKARESGSSTAEEGDFSKGPIRCDRCGYNTNRYDHYTAHLKHHTRAGDNERVYKCIICTYTTVSEYHWRKHLRNHFPRKVYTCGKCNYFSDRKNNYVQHVRTHTGERPYKCELCPYSSSQKTHLTRHMRTHSGEKPFKCDQCSYVASNQHEVTRHARQVHNGPKPLNCPHCDYKTADRSNFKKHVELHVNPRQFNCPVCDYAASKKCNLQYHFKSKHPTCPNKT

SEQ ID NO: 58 - DNA, 1104 bp, synthetic construct
  source 1..1104: mol_type = other DNA
atgaaacggacagccgatggcagcgagttcgagagccccaagaagaagagaaaggtggaattcggcagcggcttcaggtgtaaaccctgccagtacgaggccgagtctgaggaacagtttgtccaccacatcagagtgcacagcgctaagaaattcttcgttgaggaatctgccgagaagcaggccaaggcccgggaaagcggctccagtacagccgaagagggcgacttcagcaagggccctatccggtgcgacagatgtggctataataccaacagatacgaccactacacagcgcacctgaagcaccacacccgggccggcgacaacgagagagtgtacaagtgcatcatctgcacctacaccacagtgtccgagtaccactggcggaaacatctcagaaaccactttccaagaaaggtgtacacctgcggcaagtgcaactacttcagcgaccggaagaacaactacgtgcagcacgtgcggacacacaccggcgagagaccttataagtgtgaactgtgcccttacagcagcagccagaaaactcacctgacccgccacatgagaacccatagcggagaaaagccatttaagtgcgaccagtgcagctacgtggccagcaatcaacacgaggtgaccagacacgccagacaggtgcacaacggccctaagcctctgaactgtccccactgcgactacaaaaccgccgatcggagcaacttcaagaaacacgtggaactgcacgtgaatcctagacagttcaactgccccgtgtgcgattacgccgcctccaagaagtgtaacctgcaataccacttcaagagcaagcattccggcggcagcagcggaggcagcagcggcagcgagacacctggcaccagcgaatccgccacccctgagagcagcggcggctcttctggcggaagctctagagccgacgctctggacgacttcgacctggatatgctgggctccgatgctctggatgacttcgacctggacatgctgggcagcgacgccctggacgacttcgacctggacatgctgggaagcgacgccctggatgattttgatctggacatgctctacatcgacggcagc

SEQ ID NO: 59 - protein, 368 aa, synthetic construct
MKRTADGSEFESPKKKRKVEFGSGFRCKPCQYEAESEEQFVHHIRVHSAKKFFVEESAEKQAKARESGSSTAEEGDFSKGPIRCDRCGYNTNRYDHYTAHLKHHTRAGDNERVYKCIICTYTTVSEYHWRKHLRNHFPRKVYTCGKCNYFSDRKNNYVQHVRTHTGERPYKCELCPYSSSQKTHLTRHMRTHSGEKPFKCDQCSYVASNQHEVTRHARQVHNGPKPLNCPHCDYKTADRSNFKKHVELHVNPRQFNCPVCDYAASKKCNLQYHFKSKHSGGSSGGSSGSETPGTSESATPESSGGSSGGSSRADALDDFDLDMLGSDALDDFDLDMLGSDALDDFDLDMLGSDALDDFDLDMLYIDGS

SEQ ID NO: 60 - DNA, 1827 bp, synthetic construct
  source 1..1827: mol_type = other DNA
atgcctaaaaagaaaagaaaggtgggttctggtaagaccaaaccctttcgctgtaagccatgccaatatgaagcagaatctgaagaacagtttgtgcatcacatcagagttcacagtgctaagaaattttttgtggaagagagtgcagagaagcaggcaaaagccagggaatctggctcttccactgcagaagagggagatttctccaagggccccattcgctgtgaccgctgcggctacaatactaatcgatatgatcactatacagcacacctgaaacaccacaccagagctggggataatgagcgagtctacaagtgtatcatttgcacatacacaacagtgagcgagtatcactggaggaaacatttaagaaaccattttccaaggaaagtatacacatgtggaaaatgcaactatttttcagacagaaaaaacaattatgttcagcatgttagaactcatacaggagaacgcccatataaatgtgaactttgtccttactcaagttctcagaagactcatctaactagacatatgcgtactcattcaggtgagaagccatttaaatgtgatcagtgcagttatgtggcctctaatcaacatgaagtaacccgccatgcaagacaggttcacaatgggcctaaacctcttaattgcccacactgtgattacaaaacagcagatagaagcaacttcaaaaaacatgtagagctacatgtgaacccacggcagttcaattgccctgtatgtgactatgcagcttccaagaagtgtaatctacagtatcacttcaaatctaagcatcctacttgtcctaataaaacaatgggtagtggcggtggtggttcaggaggcggcggaagcccttcagggcagatcagcaaccaggccctggctctggcccctagctccgctccagtgctggcccagactatggtgccctctagtgctatggtgcctctggcccagccacctgctccagcccctgtgctgaccccaggaccaccccagtcactgagcgctccagtgcccaagtctacacaggccggcgaggggactctgagtgaagctctgctgcacctgcagttcgacgctgatgaggacctgggagctctgctggggaacagcaccgatcccggagtgttcacagatctggcctccgtggacaactctgagtttcagcagctgctgaatcagggcgtgtccatgtctcatagtacagccgaaccaatgctgatggagtaccccgaagccattacccggctggtgaccggcagccagcggccccccgaccccgctccaactcccctgggaaccagcggcctgcctaatgggctgtccggagatgaagacttctcaagcatcgctgatatggactttagtgccctgctgtcacagatttcctctagtgggcagggaggaggtggaagcggcttcagcgtggacaccagtgccctgctggacctgttcagcccctcggtgaccgtgcccgacatgagcctgcctgaccttgacagcagcctggccagtatccaagagctcctgtctccccaggagccccccaggcctcccgaggcagagaacagcagcccggattcagggaagcagctggtgcactacacagcgcagccgctgttcctgctggaccccggctccgtggacaccgggagcaacgacctgccggtgctgtttgagctgggagagggctcctacttctccgaaggggacggcttcgccgaggaccccaccatctccctgctgacaggctcggagcctcccaaagccaaggaccccactgtctcccccaagaagaagcgcaaggtg

SEQ ID NO: 61 - protein, 609 aa, synthetic construct
MPKKKRKVGSGKTKPFRCKPCQYEAESEEQFVHHIRVHSAKKFFVEESAEKQAKARESGSSTAEEGDFSKGPIRCDRCGYNTNRYDHYTAHLKHHTRAGDNERVYKCIICTYTTVSEYHWRKHLRNHFPRKVYTCGKCNYFSDRKNNYVQHVRTHTGERPYKCELCPYSSSQKTHLTRHMRTHSGEKPFKCDQCSYVASNQHEVTRHARQVHNGPKPLNCPHCDYKTADRSNFKKHVELHVNPRQFNCPVCDYAASKKCNLQYHFKSKHPTCPNKTMGSGGGGSGGGGSPSGQISNQALALAPSSAPVLAQTMVPSSAMVPLAQPPAPAPVLTPGPPQSLSAPVPKSTQAGEGTLSEALLHLQFDADEDLGALLGNSTDPGVFTDLASVDNSEFQQLLNQGVSMSHSTAEPMLMEYPEAITRLVTGSQRPPDPAPTPLGTSGLPNGLSGDEDFSSIADMDFSALLSQISSSGQGGGGSGFSVDTSALLDLFSPSVTVPDMSLPDLDSSLASIQELLSPQEPPRPPEAENSSPDSGKQLVHYTAQPLFLLDPGSVDTGSNDLPVLFELGEGSYFSEGDGFAEDPTISLLTGSEPPKAKDPTVSPKKKRKV

SEQ ID NO: 62 - DNA, 2459 bp, synthetic construct
  source 1..2459: mol_type = other DNA
ataacttacggtaaatggcccgcctggctgaccgcccaacgacccccgcccattgacgtcaataatgacgtatgttcccatagtaacgccaatagggactttccattgacgtcaatgggtggagtatttacggtaaactgcccacttggcagtacatcaagtgtatcatatgccaagtacgccccctattgacgtcaatgacggtaaatggcccgcctggcattatgcccagtacatgaccttatgggactttcctacttggcagtacatctacgtattagtcatcgctattaccatgctcgagtactagaacatatcctggtgtggagtaggggacgctgctctgacagaggctcgggggcctgagctggctctgtgagctggggaggaggcagacagccaggccttgtctgcaagcagacctggcagcattgggctggccgccccccagggcctcctcttcatgcccagtgaatgactcaccttggcacagacacaatgttcggggtgggcacagtgcctgcttcccgccgcaccccagcccccctcaaatgccttccgagaagcccattgagcagggggcttgcattgcaccccagcctgacagcctggcatcttgggataaaagcagcacagccccctaggggctgcccttgctgtgtggcgccaccggcggtggagaacaaggctctattcagcctgtgcccaggaaaggggatcaggggatgcccaggcatggacagtgggtggcagggggggagaggagggctgtctgcttcccagaagtccaaggacacaaatgggtgaggggagagctctccccatagctgggctgcggcccaaccccaccccctcaggctatgccagggggtgttgccaggggcacccgggcatcgccagtctagcccactccttcataaagccctcgcatcccaggagcgagcagagccagagcaggttggagaggagacgcatcacctccgctgctcgcgaattggatcaagaggtaagggtttaagggatggttggttggtggggtattaatgtttaattacctggagcacctgcctgaaatcactttttttcaggttggggatccgccaccatgaaacggacagccgatggcagcgagttcgagagccccaagaagaagagaaaggtgggcagcggcaagaccaagcccttcaggtgtaaaccctgccagtacgaggccgagtctgaggaacagtttgtccaccacatcagagtgcacagcgctaagaaattcttcgttgaggaatctgccgagaagcaggccaaggcccgggaaagcggctccagtacagccgaagagggcgacttcagcaagggccctatccggtgcgacagatgtggctataataccaacagatacgaccactacacagcgcacctgaagcaccacacccgggccggcgacaacgagagagtgtacaagtgcatcatctgcacctacaccacagtgtccgagtaccactggcggaaacatctcagaaaccactttccaagaaaggtgtacacctgcggcaagtgcaactacttcagcgaccggaagaacaactacgtgcagcacgtgcggacacacaccggcgagagaccttataagtgtgaactgtgcccttacagcagcagccagaaaactcacctgacccgccacatgagaacccatagcggagaaaagccatttaagtgcgaccagtgcagctacgtggccagcaatcaacacgaggtgaccagacacgccagacaggtgcacaacggccctaagcctctgaactgtccccactgcgactacaaaaccgccgatcggagcaacttcaagaaacacgtggaactgcacgtgaatcctagacagttcaactgccccgtgtgcgattacgccgcctccaagaagtgtaacctgcaataccacttcaagagcaagcatcctacatgccctaacaagaccatgggcagcaagagaacagctgatggcagcgaattcgagtcccctaagaaaaaaagaaaggtctaaataatcaacctctggattacaaaatttgtgaaagattgactggtattcttaactatgttgctccttttacgctatgtggatacgctgctttaatgcctttgtatcatgctattgcttcccgtatggctttcattttctcctccttgtataaatcctggttagttcttgccacggcggaactcatcgccgcctgccttgcccgctgctggacaggggctcggctgttgggcactgacaattccgtggtgtttatttgtgaaatttgtgatgctattgctttatttgtaaccatctagctttatttgtgaaatttgtgatgctattgctttatttgtaaccattataagctgcaataaacaagttaacaacaacaattgcattcattttatgtttcaggttcagggggagatgtgggaggttttttaaa

SEQ ID NO: 63 - protein, 276 aa, synthetic construct
MFRCKPCQYEAESEEQFVHHIRVHSAKKFFVEESAEKQAKARESGSSTAEEGDFSKGPIRCDRCGYNTNRYDHYTAHLKHHTRAGDNERVYKCIICTYTTVSEYHWRKHLRNHFPRKVYTCGKCNYFSDRKNNYVQHVRTHTGERPYKCELCPYSSSQKTHLTRHMRTHSGEKPFKCDQCSYVASNQHEVTRHARQVHNGPKPLNCPHCDYKTADRSNFKKHVELHVNPRQFNCPVCDYAASKKCNLQYHFKSKHGSGKRTADGSEFESPKKKRKV

SEQ ID NO: 64 - DNA, 795 bp, synthetic construct
  source 1..795: mol_type = other DNA
aagaccaagcccttcaggtgtaaaccctgccagtacgaggccgagtctgaggaacagtttgtccaccacatcagagtgcacagcgctaagaaattcttcgttgaggaatctgccgagaagcaggccaaggcccgggaaagcggctccagtacagccgaagagggcgacttcagcaagggccctatccggtgcgacagatgtggctataataccaacagatacgaccactacacagcgcacctgaagcaccacacccgggccggcgacaacgagagagtgtacaagtgcatcatctgcacctacaccacagtgtccgagtaccactggcggaaacatctcagaaaccactttccaagaaaggtgtacacctgcggcaagtgcaactacttcagcgaccggaagaacaactacgtgcagcacgtgcggacacacaccggcgagagaccttataagtgtgaactgtgcccttacagcagcagccagaaaactcacctgacccgccacatgagaacccatagcggagaaaagccatttaagtgcgaccagtgcagctacgtggccagcaatcaacacgaggtgaccagacacgccagacaggtgcacaacggccctaagcctctgaactgtccccactgcgactacaaaaccgccgatcggagcaacttcaagaaacacgtggaactgcacgtgaatcctagacagttcaactgccccgtgtgcgattacgccgcctccaagaagtgtaacctgcaataccacttcaagagcaagcatcctacatgccctaacaagacc

SEQ ID NO: 65 - DNA, 2209 bp, synthetic construct
  source 1..2209: mol_type = other DNA
taatcccacctccctctctgtgctgggactcacagagggagacctcaggaggcagtctgtccatcacatgtccaaatgcagagcataccctgggctgggcgcagtggcgcacaactgtaattccagcactttgggaggctgatgtggaaggatcacttgagcccagaagttctagaccagcctgggcaacatggcaagaccctatctctacaaaaaaagttaaaaaatcagccacgtgtggtgacacacacctgtagtcccagctattcaggaggctgaggtgaggggatcacttaaggctgggaggttgaggctgcagtgagtcgtggttgcgccactgcactccagcctgggcaacagtgagaccctgtctcaaaagacaaaaaaaaaaaaaaaaaaaaaagaacatatcctggtgtggagtaggggacgctgctctgacagaggctcgggggcctgagctggctctgtgagctggggaggaggcagacagccaggccttgtctgcaagcagacctggcagcattgggctggccgccccccagggcctcctcttcatgcccagtgaatgactcaccttggcacagacacaatgttcggggtgggcacagtgcctgcttcccgccgcaccccagcccccctcaaatgccttccgagaagcccattgagcagggggcttgcattgcaccccagcctgacagcctggcatcttgggataaaagcagcacagccccctaggggctgcccttgctgtgtggcgccaccggcggtggagaacaaggctctattcagcctgtgcccaggaaaggggatcaggggatgcccaggcatggacagtgggtggcagggggggagaggagggctgtctgcttcccagaagtccaaggacacaaatgggtgaggggactgggcagggttctgaccctgtgggaccagagtggagggcgtagatggacctgaagtctccagggacaacagggcccaggtctcaggctcctagttgggcccagtggctccagcgtttccaaacccatccatccccagaggttcttcccatctctccaggctgatgtgtgggaactcgaggaaataaatctccagtgggagacggaggggtggccagggaaacggggcgctgcaggaataaagacgagccagcacagccagctcatgtgtaacggctttgtggagctgtcaaggcctggtctctgggagagaggcacagggaggccagacaaggaaggggtgacctggagggacagatccaggggctaaagtcctgataaggcaagagagtgccggccccctcttgccctatcaggacctccactgccacatagaggccatgattgacccttagacaaagggctggtgtccaatcccagcccccagccccagaactccagggaatgaatgggcagagagcaggaatgtgggacatctgtgttcaagggaaggactccaggagtctgctgggaatgaggcctagtaggaaatgaggtggcccttgagggtacagaacaggttcattcttcgccaaattcccagcaccttgcaggcacttacagctgagtgagataatgcctgggttatgaaatcaaaaagttggaaagcaggtcagaggtcatctggtacagcccttccttcccttttttttttttttttttgtgagacaaggtctctctctgttgcccaggctggagtggcgcaaacacagctcactgcagcctcaacctactgggctcaagcaatcctccagcctcagcctcccaaagtgctgggattacaagcatgagccaccccactcagccctttccttcctttttaattgatgcataataattgtaagtattcatcatggtccaaccaaccctttcttgacccaccttcctagagagagggtcctcttgcttcagcggtcagggccccagacccatggtctggctccaggtaccacctgcctcatgcaggagttggcgtgcccaggaagctctgcctctgggcacagtgacctcagtggggtgaggggagctctccccatagctgggctgcggcccaaccccaccccctcaggctatgccagggggtgttgccaggggcacccgggcatcgccagtctagcccactccttcataaagccctcgcatcccaggagcgagcagagccagagcaggttggagaggagacgcatcacctccgctgctcgcgg

SEQ ID NO: 66 - DNA, 681 bp, synthetic construct
  source 1..681: mol_type = other DNA
aacatatcctggtgtggagtaggggacgctgctctgacagaggctcgggggcctgagctggctctgtgagctggggaggaggcagacagccaggccttgtctgcaagcagacctggcagcattgggctggccgccccccagggcctcctcttcatgcccagtgaatgactcaccttggcacagacacaatgttcggggtgggcacagtgcctgcttcccgccgcaccccagcccccctcaaatgccttccgagaagcccattgagcagggggcttgcattgcaccccagcctgacagcctggcatcttgggataaaagcagcacagccccctaggggctgcccttgctgtgtggcgccaccggcggtggagaacaaggctctattcagcctgtgcccaggaaaggggatcaggggatgcccaggcatggacagtgggtggcagggggggagaggagggctgtctgcttcccagaagtccaaggacacaaatgggtgaggggagagctctccccatagctgggctgcggcccaaccccaccccctcaggctatgccagggggtgttgccaggggcacccgggcatcgccagtctagcccactccttcataaagccctcgcatcccaggagcgagcagagccagagcaggttggagaggagacgcatcacctccgctgctcgc

SEQ ID NO: 67 - protein, 716 aa, synthetic construct
MRADALDDFDLDMLGSDALDDFDLDMLGSDALDDFDLDMLGSDALDDFDLDMLYIDGSGSGGSGSGSGGSGSGGSGSGKRTADGSEFESPKKKRKVGSGKTKPFRCKPCQYEAESEEQFVHHIRVHSAKKFFVEESAEKQAKARESGSSTAEEGDFSKGPIRCDRCGYNTNRYDHYTAHLKHHTRAGDNERVYKCIICTYTTVSEYHWRKHLRNHFPRKVYTCGKCNYFSDRKNNYVQHVRTHTGERPYKCELCPYSSSQKTHLTRHMRTHSGEKPFKCDQCSYVASNQHEVTRHARQVHNGPKPLNCPHCDYKTADRSNFKKHVELHVNPRQFNCPVCDYAASKKCNLQYHFKSKHPTCPNKTMGSKRTADGSEFESPKKKRKVSGGSSGGSSGSETPGTSESATPESSGGSSGGSSRADALDDFDLDMLGSDALDDFDLDMLGSDALDDFDLDMLGSDALDDFDLDMLYIDGSGSGSVLPQAPAPAPAPAMVSALAQAPAPVPVLAPGPPQAVAPPAPKPTQAGEGTLSEALLQLQFDDEDLGALLGNSTDPAVFTDLASVDNSEFQQLLNQGIPVAPHTTEPMLMEYPEAITRLVTGAQRPPDPAPAPLGAPGLPNGLLSGDEDFSSIADMDFSALLSGGGSGGSGSDLSHPPPRGHLDELTTTLESMTEDLNLDSPLTPELNEILDTFLNDECLLHAMHISTGLSIFDTSLF

SEQ ID NO: 68 - DNA, 2148 bp, synthetic construct
  source 1..2148: mol_type = other DNA
atgagagccgacgccctggatgacttcgacctggacatgctcggcagcgacgccctggacgacttcgacctggatatgctgggctccgatgctctggacgacttcgacctggacatgctgggctctgatgccctggatgattttgatctggacatgctgtacatcgacggcagcggcagcggcggcagcggcagcggcagcggcggaagcggatctggaggcagcggaagcggcaaacggacagccgatggcagcgagttcgagagccccaagaagaagagaaaggtgggcagcggcaagaccaagcccttcaggtgtaaaccctgccagtacgaggccgagtctgaggaacagtttgtccaccacatcagagtgcacagcgctaagaaattcttcgttgaggaatctgccgagaagcaggccaaggcccgggaaagcggctccagtacagccgaagagggcgacttcagcaagggccctatccggtgcgacagatgtggctataataccaacagatacgaccactacacagcgcacctgaagcaccacacccgggccggcgacaacgagagagtgtacaagtgcatcatctgcacctacaccacagtgtccgagtaccactggcggaaacatctcagaaaccactttccaagaaaggtgtacacctgcggcaagtgcaactacttcagcgaccggaagaacaactacgtgcagcacgtgcggacacacaccggcgagagaccttataagtgtgaactgtgcccttacagcagcagccagaaaactcacctgacccgccacatgagaacccatagcggagaaaagccatttaagtgcgaccagtgcagctacgtggccagcaatcaacacgaggtgaccagacacgccagacaggtgcacaacggccctaagcctctgaactgtccccactgcgactacaaaaccgccgatcggagcaacttcaagaaacacgtggaactgcacgtgaatcctagacagttcaactgccccgtgtgcgattacgccgcctccaagaagtgtaacctgcaataccacttcaagagcaagcatcctacatgccctaacaagaccatgggcagcaagcggaccgccgatggctctgagttcgagagccccaagaagaaaagaaaggtgtccggcggcagcagcggaggcagcagcggcagcgagacacctggcaccagcgaatccgccacccctgagagcagcggcggctcttctggcggaagctctagagccgacgctctggacgacttcgacctggatatgctgggctccgatgctctggatgacttcgacctggacatgctgggcagcgacgccctggacgacttcgacctggacatgctgggaagcgacgccctggatgattttgatctggacatgctctacatcgacggcagcggctctggatcagtgctgcctcaggctcctgctcctgcaccagctccagccatggtgtctgcactggctcaggcaccagcacccgtgcctgtgctggctcctggacctccacaggctgtggctccaccagcccctaaacctacacaggccggcgagggcacactgtctgaagctctgctgcagctgcagttcgacgacgaggatctgggagccctgctgggaaacagcaccgatcctgccgtgttcaccgacctggccagcgtggacaacagcgagttccagcagctgctgaaccagggcatccctgtggcccctcacaccaccgagcccatgctgatggaataccccgaggccatcacccggctcgtgacaggcgctcagaggcctcctgatccagctcctgcccctctgggagcaccaggcctgcctaatggactgctgtctggcgacgaggacttcagctctatcgccgatatggatttctcagccttgctgtcaggcggtggtagtggtgggagcggtagtgacctttcccatccgcccccaaggggccatctggatgagctgacaaccacacttgagtccatgaccgaggatctgaacctggactcacccctgaccccggaattgaacgagattctggataccttcctgaacgacgagtgcctcttgcatgccatgcatatcagcacaggactgtccatcttcgacacatctctgttt

SEQ ID NO: 69 - protein, 184 aa, synthetic construct
PSGQISNQALALAPSSAPVLAQTMVPSSAMVPLAQPPAPAPVLTPGPPQSLSAPVPKSTQAGEGTLSEALLHLQFDADEDLGALLGNSTDPGVFTDLASVDNSEFQQLLNQGVSMSHSTAEPMLMEYPEAITRLVTGSQRPPDPAPTPLGTSGLPNGLSGDEDFSSIADMDFSALLSQISSSGQ

SEQ ID NO: 70 - protein, 124 aa, synthetic construct
GFSVDTSALLDLFSPSVTVPDMSLPDLDSSLASIQELLSPQEPPRPPEAENSSPDSGKQLVHYTAQPLFLLDPGSVDTGSNDLPVLFELGEGSYFSEGDGFAEDPTISLLTGSEPPKAKDPTVS

SEQ ID NO: 71 - protein, 237 aa, synthetic construct
VLPQAPAPAPAPAMVSALAQAPAPVPVLAPGPPQAVAPPAPKPTQAGEGTLSEALLQLQFDDEDLGALLGNSTDPAVFTDLASVDNSEFQQLLNQGIPVAPHTTEPMLMEYPEAITRLVTGAQRPPDPAPAPLGAPGLPNGLLSGDEDFSSIADMDFSALLSGGGSGGSGSDLSHPPPRGHLDELTTTLESMTEDLNLDSPLTPELNEILDTFLNDECLLHAMHISTGLSIFDTSLF

SEQ ID NO: 72 - protein, 296 aa, synthetic construct
DALDDFDLDMLGSDALDDFDLDMLGSDALDDFDLDMLGSDALDDFDLDMLYIDGSGSGSVLPQAPAPAPAPAMVSALAQAPAPVPVLAPGPPQAVAPPAPKPTQAGEGTLSEALLQLQFDDEDLGALLGNSTDPAVFTDLASVDNSEFQQLLNQGIPVAPHTTEPMLMEYPEAITRLVTGAQRPPDPAPAPLGAPGLPNGLLSGDEDFSSIADMDFSALLSGGGSGGSGSDLSHPPPRGHLDELTTTLESMTEDLNLDSPLTPELNEILDTFLNDECLLHAMHISTGLSIFDTSLF

SEQ ID NO: 73 - protein, 380 aa, synthetic construct
DALDDFDLDMLGSDALDDFDLDMLGSDALDDFDLDMLGSDALDDFDLDMLYIDGSGSGGGGSGGGGSPSGQISNQALALAPSSAPVLAQTMVPSSAMVPLAQPPAPAPVLTPGPPQSLSAPVPKSTQAGEGTLSEALLHLQFDADEDLGALLGNSTDPGVFTDLASVDNSEFQQLLNQGVSMSHSTAEPMLMEYPEAITRLVTGSQRPPDPAPTPLGTSGLPNGLSGDEDFSSIADMDFSALLSQISSSGQGGGGSGFSVDTSALLDLFSPSVTVPDMSLPDLDSSLASIQELLSPQEPPRPPEAENSSPDSGKQLVHYTAQPLFLLDPGSVDTGSNDLPVLFELGEGSYFSEGDGFAEDPTISLLTGSEPPKAKDPTVS

SEQ ID NO: 74 - protein, 204 aa, synthetic construct
GDFSKGPIRCDRCGYNTNRYDHYTAHLKHHTRAGDNERVYKCIICTYTTVSEYHWRKHLRNHFPRKVYTCGKCNYFSDRKNNYVQHVRTHTGERPYKCELCPYSSSQKTHLTRHMRTHSGEKPFKCDQCSYVASNQHEVTRHARQVHNGPKPLNCPHCDYKTADRSNFKKHVELHVNPRQFNCPVCDYAASKKCNLQYHFKSKH

SEQ ID NO: 75 - protein, 230 aa, synthetic construct
FRCKPCQYEAESEEQFVHHIRVHSAKKFFVEESAEKQAKARESGSSTAEEGDFSKGPIRCDRCGYNTNRYDHYTAHLKHHTRAGDNERVYKCIICTYTTVSEYHWRKHLRNHFPRKVYTCGKCNYFSDRKNNYVQHVRTHTGERPYKCELCPYSSSQKTHLTRHMRTHSGEKPFKCDQCSYVASNQHEVTRHARQVHNGPKPLNCPHCDYKTADRSNFKKHVELHVNPRQ

SEQ ID NO: 76 - protein, 180 aa, synthetic construct
GDFSKGPIRCDRCGYNTNRYDHYTAHLKHHTRAGDNERVYKCIICTYTTVSEYHWRKHLRNHFPRKVYTCGKCNYFSDRKNNYVQHVRTHTGERPYKCELCPYSSSQKTHLTRHMRTHSGEKPFKCDQCSYVASNQHEVTRHARQVHNGPKPLNCPHCDYKTADRSNFKKHVELHVNPRQ

SEQ ID NO: 77 - protein, 254 aa, synthetic construct; identical to SEQ ID NO: 2

SEQ ID NO: 78 - protein, 226 aa, synthetic construct
MKRTADGSEFESPKKKRKVGSGGDFSKGPIRCDRCGYNTNRYDHYTAHLKHHTRAGDNERVYKCIICTYTTVSEYHWRKHLRNHFPRKVYTCGKCNYFSDRKNNYVQHVRTHTGERPYKCELCPYSSSQKTHLTRHMRTHSGEKPFKCDQCSYVASNQHEVTRHARQVHNGPKPLNCPHCDYKTADRSNFKKHVELHVNPRQFNCPVCDYAASKKCNLQYHFKSKH

SEQ ID NO: 79 - protein, 252 aa, synthetic construct
MKRTADGSEFESPKKKRKVGSGFRCKPCQYEAESEEQFVHHIRVHSAKKFFVEESAEKQAKARESGSSTAEEGDFSKGPIRCDRCGYNTNRYDHYTAHLKHHTRAGDNERVYKCIICTYTTVSEYHWRKHLRNHFPRKVYTCGKCNYFSDRKNNYVQHVRTHTGERPYKCELCPYSSSQKTHLTRHMRTHSGEKPFKCDQCSYVASNQHEVTRHARQVHNGPKPLNCPHCDYKTADRSNFKKHVELHVNPRQ

SEQ ID NO: 80 - protein, 202 aa, synthetic construct
MKRTADGSEFESPKKKRKVGSGGDFSKGPIRCDRCGYNTNRYDHYTAHLKHHTRAGDNERVYKCIICTYTTVSEYHWRKHLRNHFPRKVYTCGKCNYFSDRKNNYVQHVRTHTGERPYKCELCPYSSSQKTHLTRHMRTHSGEKPFKCDQCSYVASNQHEVTRHARQVHNGPKPLNCPHCDYKTADRSNFKKHVELHVNPRQ

SEQ ID NO: 81 - protein, 723 aa, synthetic construct
MKRTADGSEFESPKKKRKVGSGKTKPFRCKPCQYEAESEEQFVHHIRVHSAKKFFVEESAEKQAKARESGSSTAEEGDFSKGPIRCDRCGYNTNRYDHYTAHLKHHTRAGDNERVYKCIICTYTTVSEYHWRKHLRNHFPRKVYTCGKCNYFSDRKNNYVQHVRTHTGERPYKCELCPYSSSQKTHLTRHMRTHSGEKPFKCDQCSYVASNQHEVTRHARQVHNGPKPLNCPHCDYKTADRSNFKKHVELHVNPRQFNCPVCDYAASKKCNLQYHFKSKHPTCPNKTMGSKRTADGSEFESPKKKRKVSGGSSGGSSGSETPGTSESATPESSGGSSGGSSRADALDDFDLDMLGSDALDDFDLDMLGSDALDDFDLDMLGSDALDDFDLDMLYIDGSGSGGGGSGGGGSPSGQISNQALALAPSSAPVLAQTMVPSSAMVPLAQPPAPAPVLTPGPPQSLSAPVPKSTQAGEGTLSEALLHLQFDADEDLGALLGNSTDPGVFTDLASVDNSEFQQLLNQGVSMSHSTAEPMLMEYPEAITRLVTGSQRPPDPAPTPLGTSGLPNGLSGDEDFSSIADMDFSALLSQISSSGQGGGGSGFSVDTSALLDLFSPSVTVPDMSLPDLDSSLASIQELLSPQEPPRPPEAENSSPDSGKQLVHYTAQPLFLLDPGSVDTGSNDLPVLFELGEGSYFSEGDGFAEDPTISLLTGSEPPKAKDPTVS

SEQ ID NO: 82 - protein, 639 aa, synthetic construct
MKRTADGSEFESPKKKRKVGSGKTKPFRCKPCQYEAESEEQFVHHIRVHSAKKFFVEESAEKQAKARESGSSTAEEGDFSKGPIRCDRCGYNTNRYDHYTAHLKHHTRAGDNERVYKCIICTYTTVSEYHWRKHLRNHFPRKVYTCGKCNYFSDRKNNYVQHVRTHTGERPYKCELCPYSSSQKTHLTRHMRTHSGEKPFKCDQCSYVASNQHEVTRHARQVHNGPKPLNCPHCDYKTADRSNFKKHVELHVNPRQFNCPVCDYAASKKCNLQYHFKSKHPTCPNKTMGSKRTADGSEFESPKKKRKVSGGSSGGSSGSETPGTSESATPESSGGSSGGSSRADALDDFDLDMLGSDALDDFDLDMLGSDALDDFDLDMLGSDALDDFDLDMLYIDGSGSGSVLPQAPAPAPAPAMVSALAQAPAPVPVLAPGPPQAVAPPAPKPTQAGEGTLSEALLQLQFDDEDLGALLGNSTDPAVFTDLASVDNSEFQQLLNQGIPVAPHTTEPMLMEYPEAITRLVTGAQRPPDPAPAPLGAPGLPNGLLSGDEDFSSIADMDFSALLSGGGSGGSGSDLSHPPPRGHLDELTTTLESMTEDLNLDSPLTPELNEILDTFLNDECLLHAMHISTGLSIFDTSLF

SEQ ID NO: 83 - RNA, 30 nt, synthetic construct
  source 1..30: mol_type = other RNA
ttctggaagttcttggagcccggcttcttg

SEQ ID NO: 84 - protein, 723 aa, synthetic construct; identical to SEQ ID NO: 81

SEQ ID NO: 85 - DNA, 2169 bp, synthetic construct
  source 1..2169: mol_type = other DNA
atgaaacggacagccgatggcagcgagttcgagagccccaagaagaagagaaaggtgggcagcggcaagaccaagcccttcaggtgtaaaccctgccagtacgaggccgagtctgaggaacagtttgtccaccacatcagagtgcacagcgctaagaaattcttcgttgaggaatctgccgagaagcaggccaaggcccgggaaagcggctccagtacagccgaagagggcgacttcagcaagggccctatccggtgcgacagatgtggctataataccaacagatacgaccactacacagcgcacctgaagcaccacacccgggccggcgacaacgagagagtgtacaagtgcatcatctgcacctacaccacagtgtccgagtaccactggcggaaacatctcagaaaccactttccaagaaaggtgtacacctgcggcaagtgcaactacttcagcgaccggaagaacaactacgtgcagcacgtgcggacacacaccggcgagagaccttataagtgtgaactgtgcccttacagcagcagccagaaaactcacctgacccgccacatgagaacccatagcggagaaaagccatttaagtgcgaccagtgcagctacgtggccagcaatcaacacgaggtgaccagacacgccagacaggtgcacaacggccctaagcctctgaactgtccccactgcgactacaaaaccgccgatcggagcaacttcaagaaacacgtggaactgcacgtgaatcctagacagttcaactgccccgtgtgcgattacgccgcctccaagaagtgtaacctgcaataccacttcaagagcaagcatcctacatgccctaacaagaccatgggcagcaagcggaccgccgatggctctgagttcgagagccccaagaagaaaagaaaggtgtccggcggcagcagcggaggcagcagcggcagcgagacacctggcaccagcgaatccgccacccctgagagcagcggcggctcttctggcggaagctctagagccgacgctctggacgacttcgacctggatatgctgggctccgatgctctggatgacttcgacctggacatgctgggcagcgacgccctggacgacttcgacctggacatgctgggaagcgacgccctggatgattttgatctggacatgctctacatcgacggcagcggtagtggcggtggtggttcaggaggcggcggaagcccttcagggcagatcagcaaccaggccctggctctggcccctagctccgctccagtgctggcccagactatggtgccctctagtgctatggtgcctctggcccagccacctgctccagcccctgtgctgaccccaggaccaccccagtcactgagcgctccagtgcccaagtctacacaggccggcgaggggactctgagtgaagctctgctgcacctgcagttcgacgctgatgaggacctgggagctctgctggggaacagcaccgatcccggagtgttcacagatctggcctccgtggacaactctgagtttcagcagctgctgaatcagggcgtgtccatgtctcatagtacagccgaaccaatgctgatggagtaccccgaagccattacccggctggtgaccggcagccagcggccccccgaccccgctccaactcccctgggaaccagcggcctgcctaatgggctgtccggagatgaagacttctcaagcatcgctgatatggactttagtgccctgctgtcacagatttcctctagtgggcagggaggaggtggaagcggcttcagcgtggacaccagtgccctgctggacctgttcagcccctcggtgaccgtgcccgacatgagcctgcctgaccttgacagcagcctggccagtatccaagagctcctgtctccccaggagccccccaggcctcccgaggcagagaacagcagcccggattcagggaagcagctggtgcactacacagcgcagccgctgttcctgctggaccccggctccgtggacaccgggagcaacgacctgccggtgctgtttgagctgggagagggctcctacttctccgaaggggacggcttcgccgaggaccccaccatctccctgctgacaggctcggagcctcccaaagccaaggaccccactgtctcc

SEQ ID NO: 86 - protein, 639 aa, synthetic construct; identical to SEQ ID NO: 82

SEQ ID NO: 87 - DNA, 1917 bp, synthetic construct
  source 1..1917: mol_type = other DNA
atgaaacggacagccgatggcagcgagttcgagagccccaagaagaagagaaaggtgggcagcggcaagaccaagcccttcaggtgtaaaccctgccagtacgaggccgagtctgaggaacagtttgtccaccacatcagagtgcacagcgctaagaaattcttcgttgaggaatctgccgagaagcaggccaaggcccgggaaagcggctccagtacagccgaagagggcgacttcagcaagggccctatccggtgcgacagatgtggctataataccaacagatacgaccactacacagcgcacctgaagcaccacacccgggccggcgacaacgagagagtgtacaagtgcatcatctgcacctacaccacagtgtccgagtaccactggcggaaacatctcagaaaccactttccaagaaaggtgtacacctgcggcaagtgcaactacttcagcgaccggaagaacaactacgtgcagcacgtgcggacacacaccggcgagagaccttataagtgtgaactgtgcccttacagcagcagccagaaaactcacctgacccgccacatgagaacccatagcggagaaaagccatttaagtgcgaccagtgcagctacgtggccagcaatcaacacgaggtgaccagacacgccagacaggtgcacaacggccctaagcctctgaactgtccccactgcgactacaaaaccgccgatcggagcaacttcaagaaacacgtggaactgcacgtgaatcctagacagttcaactgccccgtgtgcgattacgccgcctccaagaagtgtaacctgcaataccacttcaagagcaagcatcctacatgccctaacaagaccatgggcagcaagcggaccgccgatggctctgagttcgagagccccaagaagaaaagaaaggtgtccggcggcagcagcggaggcagcagcggcagcgagacacctggcaccagcgaatccgccacccctgagagcagcggcggctcttctggcggaagctctagagccgacgctctggacgacttcgacctggatatgctgggctccgatgctctggatgacttcgacctggacatgctgggcagcgacgccctggacgacttcgacctggacatgctgggaagcgacgccctggatgattttgatctggacatgctctacatcgacggcagcggctctggatcagtgctgcctcaggctcctgctcctgcaccagctccagccatggtgtctgcactggctcaggcaccagcacccgtgcctgtgctggctcctggacctccacaggctgtggctccaccagcccctaaacctacacaggccggcgagggcacactgtctgaagctctgctgcagctgcagttcgacgacgaggatctgggagccctgctgggaaacagcaccgatcctgccgtgttcaccgacctggccagcgtggacaacagcgagttccagcagctgctgaaccagggcatccctgtggcccctcacaccaccgagcccatgctgatggaataccccgaggccatcacccggctcgtgacaggcgctcagaggcctcctgatccagctcctgcccctctgggagcaccaggcctgcctaatggactgctgtctggcgacgaggacttcagctctatcgccgatatggatttctcagccttgctgtcaggcggtggtagtggtgggagcggtagtgacctttcccatccgcccccaaggggccatctggatgagctgacaaccacacttgagtccatgaccgaggatctgaacctggactcacccctgaccccggaattgaacgagattctggataccttcctgaacgacgagtgcctcttgcatgccatgcatatcagcacaggactgtccatcttcgacacatctctgttt

SEQ ID NO: 88 - protein, 992 aa, synthetic construct
MFSDSEEGEGLEESADIKGEPHGLENMELRSLELSVVEPQPVFEASGAPDIYSSNKDLPPETPGAEDKGKSSKTKPFRCKPCQYEAESEEQFVHHIRVHSAKKFFVEESAEKQAKARESGSSTAEEGDFSKGPIRCDRCGYNTNRYDHYTAHLKHHTRAGDNERVYKCIICTYTTVSEYHWRKHLRNHFPRKVYTCGKCNYFSDRKNNYVQHVRTHTGERPYKCELCPYSSSQKTHLTRHMRTHSGEKPFKCDQCSYVASNQHEVTRHARQVHNGPKPLNCPHCDYKTADRSNFKKHVELHVNPRQFNCPVCDYAASKKCNLQYHFKSKHPTCPNKTMDVSKVKLKKTKKREADLPDNITNEKTEIEQTKIKGDVAGKKNEKSVKAEKRDVSKEKKPSNNVSVIQVTTRTRKSVTEVKEMDVHTGSNSEKFSKTKKSKRKLEVDSHSLHGPVNDEESSTKKKKKVESKSKNNSQEVPKGDSKVEENKKQNTCMKKSTKKKTLKNKSSKKSSKPPQKEPVEKGSAQMDPPQMGPAPTEAVQKGPVQVEPPPPMEHAQMEGAQIRPAPDEPVQMEVVQEGPAQKELLPPVEPAQMVGAQIVLAHMELPPPMETAQTEVAQMGPAPMEPAQMEVAQVESAPMQVVQKEPVQMELSPPMEVVQKEPVQIELSPPMEVVQKEPVKIELSPPIEVVQKEPVQMELSPPMGVVQKEPAQREPPPPREPPLHMEPISKKPPLRKDKKEKSNMQSERARKEQVLIEVGLVPVKDSWLLKESVSTEDLSPPSPPLPKENLREEASGDQKLLNTGEGNKEAPLQKVGAEEADESLPGLAANINESTHISSSGQNLNTPEGETLNGKHQTDSIVCEMKMDTDQNTRENLTGINSTVEEPVSPMLPPSAVEEREAVSKTALASPPATMAANESQEIDEGSGGGGSGGGGSRADALDDFDLDMLGSDALDDFDLDMLGSDALDDFDLDMLGSDALDDFDLDMLYID

SEQ ID NO: 89 - protein, 449 aa, synthetic construct
MAELMPVGDNNFSDSEEGEGLEESADIKGEPHGLENMELRSLELSVVEPQPVFEASGAPDIYSSNKDLPPETPGAEDKGKSSKTKPFRCKPCQYEAESEEQFVHHIRVHSAKKFFVEESAEKQAKARESGSSTAEEGDFSKGPIRCDRCGYNTNRYDHYTAHLKHHTRAGDNERVYKCIICTYTTVSEYHWRKHLRNHFPRKVYTCGKCNYFSDRKNNYVQHVRTHTGERPYKCELCPYSSSQKTHLTRHMRTHSGEKPFKCDQCSYVASNQHEVTRHARQVHNGPKPLNCPHCDYKTADRSNFKKHVELHVNPRQFNCPVCDYAASKKCNLQYHFKSKHPTCPNKTMDVSKVKLKKTKKREADLPDNITNEKTEIEQTKIKGDVAGKKNEKSVKAEKRDVSKEKKPSNNVSVIQVTTRTRKSVTEVKEMDVHTGSGSDALDDFDLDML

SEQ ID NO: 90 - protein, 398 aa, synthetic construct
MKRTADGSEFESPKKKRKVGSGKTKPFRCKPCQYEAESEEQFVHHIRVHSAKKFFVEESAEKQAKARESGSSTAEEGDFSKGPIRCDRCGYNTNRYDHYTAHLKHHTRAGDNERVYKCIICTYTTVSEYHWRKHLRNHFPRKVYTCGKCNYFSDRKNNYVQHVRTHTGERPYKCELCPYSSSQKTHLTRHMRTHSGEKPFKCDQCSYVASNQHEVTRHARQVHNGPKPLNCPHCDYKTADRSNFKKHVELHVNPRQFNCPVCDYAASKKCNLQYHFKSKHPTCPNKTMGSKRTADGSEFESPKKKRKVSGGSSGGSSGSETPGTSESATPESSGGSSGGSSRADALDDFDLDMLGSDALDDFDLDMLGSDALDDFDLDMLGSDALDDFDLDMLYIDGS

SEQ ID NO: 91 - DNA, 1194 bp, synthetic construct
  source 1..1194: mol_type = other DNA
atgaaacggacagccgatggcagcgagttcgagagccccaagaagaagagaaaggtgggcagcggcaagaccaagcccttcaggtgtaaaccctgccagtacgaggccgagtctgaggaacagtttgtccaccacatcagagtgcacagcgctaagaaattcttcgttgaggaatctgccgagaagcaggccaaggcccgggaaagcggctccagtacagccgaagagggcgacttcagcaagggccctatccggtgcgacagatgtggctataataccaacagatacgaccactacacagcgcacctgaagcaccacacccgggccggcgacaacgagagagtgtacaagtgcatcatctgcacctacaccacagtgtccgagtaccactggcggaaacatctcagaaaccactttccaagaaaggtgtacacctgcggcaagtgcaactacttcagcgaccggaagaacaactacgtgcagcacgtgcggacacacaccggcgagagaccttataagtgtgaactgtgcccttacagcagcagccagaaaactcacctgacccgccacatgagaacccatagcggagaaaagccatttaagtgcgaccagtgcagctacgtggccagcaatcaacacgaggtgaccagacacgccagacaggtgcacaacggccctaagcctctgaactgtccccactgcgactacaaaaccgccgatcggagcaacttcaagaaacacgtggaactgcacgtgaatcctagacagttcaactgccccgtgtgcgattacgccgcctccaagaagtgtaacctgcaataccacttcaagagcaagcatcctacatgccctaacaagaccatgggcagcaagcggaccgccgatggctctgagttcgagagccccaagaagaaaagaaaggtgtccggcggcagcagcggaggcagcagcggcagcgagacacctggcaccagcgaatccgccacccctgagagcagcggcggctcttctggcggaagctctagagccgacgctctggacgacttcgacctggatatgctgggctccgatgctctggatgacttcgacctggacatgctgggcagcgacgccctggacgacttcgacctggacatgctgggaagcgacgccctggatgattttgatctggacatgctctacatcgacggcagc

SEQ ID NO: 92 - protein, 486 aa, synthetic construct
MKRTADGSEFESPKKKRKVGSGDALDDFDLDMLGSDALDDFDLDMLGSDALDDFDLDMLGSDALDDFDLDMLYIDGSSGGSSGGSSGSETPGTSESATPESSGGSSGGSSKTKPFRCKPCQYEAESEEQFVHHIRVHSAKKFFVEESAEKQAKARESGSSTAEEGDFSKGPIRCDRCGYNTNRYDHYTAHLKHHTRAGDNERVYKCIICTYTTVSEYHWRKHLRNHFPRKVYTCGKCNYFSDRKNNYVQHVRTHTGERPYKCELCPYSSSQKTHLTRHMRTHSGEKPFKCDQCSYVASNQHEVTRHARQVHNGPKPLNCPHCDYKTADRSNFKKHVELHVNPRQFNCPVCDYAASKKCNLQYHFKSKHPTCPNKTMSGGSSGGSSGSETPGTSESATPESSGGSSGGSSRADALDDFDLDMLGSDALDDFDLDMLGSDALDDFDLDMLGSDALDDFDLDMLYIDGSGSKRTADGSEFESPKKKRKV

SEQ ID NO: 93 - DNA, 1458 bp, synthetic construct
  source 1..1458: mol_type = other DNA
atgaaacggacagccgatggcagcgagttcgagagccccaagaagaagagaaaggtgggcagcggcgacgctctggacgacttcgacctggatatgctgggctccgatgctctggatgacttcgacctggacatgctgggcagcgacgccctggacgacttcgacctggacatgctgggaagcgacgccctggatgattttgatctggacatgctctacatcgacggcagctccggcggcagcagcggaggcagcagcggcagcgagacacctggcaccagcgaatccgccacccctgagagcagcggcggctcttctggcggaagctctaagaccaagcccttcaggtgtaaaccctgccagtacgaggccgagtctgaggaacagtttgtccaccacatcagagtgcacagcgctaagaaattcttcgttgaggaatctgccgagaagcaggccaaggcccgggaaagcggctccagtacagccgaagagggcgacttcagcaagggccctatccggtgcgacagatgtggctataataccaacagatacgaccactacacagcgcacctgaagcaccacacccgggccggcgacaacgagagagtgtacaagtgcatcatctgcacctacaccacagtgtccgagtaccactggcggaaacatctcagaaaccactttccaagaaaggtgtacacctgcggcaagtgcaactacttcagcgaccggaagaacaactacgtgcagcacgtgcggacacacaccggcgagagaccttataagtgtgaactgtgcccttacagcagcagccagaaaactcacctgacccgccacatgagaacccatagcggagaaaagccatttaagtgcgaccagtgcagctacgtggccagcaatcaacacgaggtgaccagacacgccagacaggtgcacaacggccctaagcctctgaactgtccccactgcgactacaaaaccgccgatcggagcaacttcaagaaacacgtggaactgcacgtgaatcctagacagttcaactgccccgtgtgcgattacgccgcctccaagaagtgtaacctgcaataccacttcaagagcaagcatcctacatgccctaacaagaccatgtccggcggcagcagcggaggcagcagcggcagcgagacacctggcaccagcgaatccgccacccctgagagcagcggcggctcttctggcggaagctctagagccgacgctctggacgacttcgacctggatatgctgggctccgatgctctggatgacttcgacctggacatgctgggcagcgacgccctggacgacttcgacctggacatgctgggaagcgacgccctggatgattttgatctggacatgctctacatcgacggcagcggcagcaagcggaccgccgatggctctgagttcgagagccccaagaagaaaagaaaggtg

SEQ ID NO: 94 - DNA, 2976 bp, synthetic construct
  source 1..2976: mol_type = other DNA
atgttttcagatagtgaagaaggagaaggacttgaagagtctgctgatataaaaggtgaacctcatggactggaaaacatggaactgagaagtttggaactcagcgtcgtagaacctcagcctgtatttgaggcatcaggtgctccagatatttacagttcaaataaagatcttccccctgaaacacctggagcggaggacaaaggcaagagctcgaagaccaaaccctttcgctgtaagccatgccaatatgaagcagaatctgaagaacagtttgtgcatcacatcagagttcacagtgctaagaaattttttgtggaagagagtgcagagaagcaggcaaaagccagggaatctggctcttccactgcagaagagggagatttctccaagggccccattcgctgtgaccgctgcggctacaatactaatcgatatgatcactatacagcacacctgaaacaccacaccagagctggggataatgagcgagtctacaagtgtatcatttgcacatacacaacagtgagcgagtatcactggaggaaacatttaagaaaccattttccaaggaaagtatacacatgtggaaaatgcaactatttttcagacagaaaaaacaattatgttcagcatgttagaactcatacaggagaacgcccatataaatgtgaactttgtccttactcaagttctcagaagactcatctaactagacatatgcgtactcattcaggtgagaagccatttaaatgtgatcagtgcagttatgtggcctctaatcaacatgaagtaacccgccatgcaagacaggttcacaatgggcctaaacctcttaattgcccacactgtgattacaaaacagcagatagaagcaacttcaaaaaacatgtagagctacatgtgaacccacggcagttcaattgccctgtatgtgactatgcagcttccaagaagtgtaatctacagtatcacttcaaatctaagcatcctacttgtcctaataaaacaatggatgtctcaaaagtgaaactaaagaaaaccaaaaaacgagaggctgacttgcctgataatattaccaatgaaaaaacagaaatagaacaaacaaaaataaaaggggatgtggctggaaagaaaaatgaaaagtccgtcaaagcagagaaaagagatgtctcaaaagagaaaaagccttctaataatgtgtcagtgatccaggtgactaccagaactcgaaaatcagtaacagaggtgaaagagatggatgtgcatacaggaagcaattcagaaaaattcagtaaaactaagaaaagcaaaaggaagctggaagttgacagccattctttacatggtcctgtgaatgatgaggaatcttcaacaaaaaagaaaaagaaggtagaaagcaaatccaaaaataatagtcaggaagtgccaaagggtgacagcaaagtggaggagaataaaaagcaaaatacttgcatgaaaaaaagtacaaagaagaaaactctgaaaaataaatcaagtaagaaaagcagtaagcctcctcagaaggaacctgttgagaagggatctgctcagatggaccctcctcagatggggcctgctcccacagaggcggttcagaaggggcccgttcaggtggagccgccacctcccatggagcatgctcagatggagggtgcccagatacggcctgctcctgacgagcctgttcagatggaggtggttcaggaggggcctgctcagaaggagctgctgcctcccgtggagcctgctcagatggtgggtgcccaaattgtacttgctcacatggagctgcctcctcccatggagactgctcagacggaggttgcccaaatggggcctgctcccatggaacctgctcagatggaggttgcccaggtagaatctgctcccatgcaggtggtccagaaggagcctgttcagatggagctgtctcctcccatggaggtggtccagaaggagcctgttcagatagagctgtctcctcccatggaggtggtccagaaggaacctgttaagatagagctgtctcctcccatagaggtggtccagaaggagcctgttcagatggagttgtctcctcccatgggggtggttcagaaggagcctgctcagagggagccacctcctcccagagagcctccccttcacatggagccaatttccaaaaagcctcctctccgaaaagataaaaaggaaaagtctaacatgcagagtgaaagggcacggaaggagcaagtccttattgaagttggcttagtgcctgttaaagatagctggcttctaaaggaaagtgtaagcacagaggatctctcaccaccatcaccaccactgccaaaggaaaatttaagagaagaggcatcaggagaccaaaaattactcaacacaggtgaaggaaataaagaagcccctcttcagaaagtaggagcagaagaggcagatgagagcctacctggtcttgctgctaatatcaacgaatctacccatatttcatcctctggacaaaacttgaatacgccagagggtgaaactttaaatggtaaacatcagactgacagtatagtttgtgaaatgaaaatggacactgatcagaacacaagagagaatctcactggtataaattcaacagttgaagaaccagtttcaccaatgcttcccccttcagcagtagaagaacgtgaagcagtgtccaaaactgcactggcatcacctcctgctacaatggcagcaaatgagtctcaggaaattgatgaaggtagtggcggtggtggttcaggaggcggcggaagccgcgccgacgcgctggacgatttcgatctcgacatgctgggttctgatgccctcgatgactttgacctggatatgttgggaagcgacgcattggatgactttgatctggacatgctcggctccgatgctctggacgatttcgatctcgatatgttatatatcgat

SEQ ID NO: 95 - DNA, 1347 bp, synthetic construct
  source 1..1347: mol_type = other DNA
atggcagaactgatgccggttggggataacaacttttcagatagtgaagaaggagaaggacttgaagagtctgctgatataaaaggtgaacctcatggactggaaaacatggaactgagaagtttggaactcagcgtcgtagaacctcagcctgtatttgaggcatcaggtgctccagatatttacagttcaaataaagatcttccccctgaaacacctggagcggaggacaaaggcaagagctcgaagaccaaaccctttcgctgtaagccatgccaatatgaagcagaatctgaagaacagtttgtgcatcacatcagagttcacagtgctaagaaattttttgtggaagagagtgcagagaagcaggcaaaagccagggaatctggctcttccactgcagaagagggagatttctccaagggccccattcgctgtgaccgctgcggctacaatactaatcgatatgatcactatacagcacacctgaaacaccacaccagagctggggataatgagcgagtctacaagtgtatcatttgcacatacacaacagtgagcgagtatcactggaggaaacatttaagaaaccattttccaaggaaagtatacacatgtggaaaatgcaactatttttcagacagaaaaaacaattatgttcagcatgttagaactcatacaggagaacgcccatataaatgtgaactttgtccttactcaagttctcagaagactcatctaactagacatatgcgtactcattcaggtgagaagccatttaaatgtgatcagtgcagttatgtggcctctaatcaacatgaagtaacccgccatgcaagacaggttcacaatgggcctaaacctcttaattgcccacactgtgattacaaaacagcagatagaagcaacttcaaaaaacatgtagagctacatgtgaacccacggcagttcaattgccctgtatgtgactatgcagcttccaagaagtgtaatctacagtatcacttcaaatctaagcatcctacttgtcctaataaaacaatggatgtctcaaaagtgaaactaaagaaaaccaaaaaacgagaggctgacttgcctgataatattaccaatgaaaaaacagaaatagaacaaacaaaaataaaaggggatgtggctggaaagaaaaatgaaaagtccgtcaaagcagagaaaagagatgtctcaaaagagaaaaagccttctaataatgtgtcagtgatccaggtgactaccagaactcgaaaatcagtaacagaggtgaaagagatggatgtgcatacaggaagcggctccgatgctctggacgacttcgacctggacatgctg